European Patent Specification EP 3 765 856 B1, published September 27, 2023. Title: METHODS FOR THE PREPARATION OF TRYPSIN-RESISTANT POLYPEPTIDES FOR MASS SPECTROMETRIC ANALYSIS. Applicant: Amgen Inc. Benchaar, Sabrina Dykstra, Andrew. The sequence listing filed with the application follows.

SEQUENCE LISTING (87 sequences)

SEQ ID NO: 1 - protein, 267 aa, Homo sapiens
  SIGNAL (1)..(27)
  PROPEP (28)..(29)
  mat_peptide (30)..(267)
  DOMAIN (30)..(247): peptidase S1 domain
MTLGRRLACLFLACVLPALLLGGTALASEIVGGRRARPHAWPFMVSLQLRGGHFCGATLIAPNFVMSAAHCVANVNVRAVRVVLGAHNLSRREPTRQVFAVQRIFENGYDPVNLLNDIVILQLNGSATINANVQVAQLPAQGRRLGNGVQCLAMGWGLLGRNRGIASVLQELNVTVVTSLCRRSNVCTLVRGRQAGVCFGDSGSPLVCNGLIHGIASFVRGGCASGLYPDAFAPVAQFVNWIDSIIQRSEDNPCPHPRDPDPASRTH

SEQ ID NO: 2 - protein, 239 aa, Homo sapiens
MRLPAQLLGLLMLWVPGSSGDIVMTQTPLSSPVTLGQPASISCRSSQSLVHSDGNTYLNWLQQRPGQPPRLLIYKISNRFSGVPDRFTGSGAGTDFTLKISRVEAEDVGVYTCMQVTQFPLTFGQGTRLEIKRTVAAPSVFIFPPSDEQLKSGTASVVCLLNNFYPREAKVQWKVDNALQSGNSQESVTEQDSKDSTYSLSSTLTLSKADYEKHKVYACEVTHQGLSSPVTKSFNRGEC

SEQ ID NO: 3 - protein, 470 aa, Homo sapiens [sequence omitted]

SEQ ID NO: 4 - protein, 235 aa, Homo sapiens
METPAQLLFLLLLWLPDTTGEIVLTQSPGTLSLSPGDRATLSCRASQSVSSSYFAWYQQKPGQAPRLLIYGASSRATGIPDRFSGSGSGTDFTLTISRLEPEDFAVYYCQQYDRSPRTFGQGTKVEIKRTVAAPSVFIFPPSDEQLKSGTASVVCLLNNFYPREAKVQWKVDNALQSGNSQESVTEQDSKDSTYSLSSTLTLSKADYEKHKVYACEVTHQGLSSPVTKSFNRGEC

SEQ ID NO: 5 - protein, 463 aa, Homo sapiens
MDWTWRILFLVAAATGAHSQVQLVQSGAEVKKPGASVKVSCKSSGYTFTGYYMHWVRQAPGQGLEWMGWINPNSGGTNYAQKFKGRVTMTRDTSISTAYMELSRLRSDDTAVYYCARDKWLDGFDYWGQGTLVTVSSASTKGPSVFPLAPCSRSTSESTAALGCLVKDYFPEPVTVSWNSGALTSGVHTFPAVLQSSGLYSLSSVVTVPSSNFGTQTYTCNVDHKPSNTKVDKTVERKCCVECPPCPAPPVAGPSVFLFPPKPKDTLMISRTPEVTCVVVDVSHEDPEVQFNWYVDGVEVHNAKTKPREEQFNSTFRVVSVLTVVHQDWLNGKEYKCKVSNKGLPAPIEKTISKTKGQPREPQVYTLPPSREEMTKNQVSLTCLVKGFYPSDIAVEWESNGQPENNYKTTPPMLDSDGSFFLYSKLTVDKSRWQQGNVFSCSVMHEALHNHYTQKSLSLSPGK

SEQ ID NO: 6 - protein, 235 aa, Homo sapiens
MAWALLLLTLLTQDTGSWAQSVLTQSPSASGTPGQRVTISCSGSSSNIGSNYVYWYQQLPGAAPKLLILRNNQRPSGVPDRFSGSKSGTSASLTISGLRSEDEADYYCAAWDDSLSGWVFGGGTKLTVLGQPKANPTVTLFPPSSEELQANKATLVCLISDFYPGAVTVAWKADGSPVKAGVETTKPSKQSNNKYAASSYLSLTPEQWKSHRSYSCQVTHEGSTVEKTVAPTECS

SEQ ID NO: 7 - protein, 479 aa, Homo sapiens
MDMRVPAQLLGLLLLWLRGARCEVQLVESGGGLVKPGGSLRLSCAASGFTFSNAWMSWVRQAPGKGLEWVGRIKSKTDGGTTDYTAPVKGRFTISRDDSKNTLYLQMNSLKAEDTAVYYCTTDRTGYSISWSSYYYYYGMDVWGQGTTVTVSSASTKGPSVFPLAPCSRSTSESTAALGCLVKDYFPEPVTVSWNSGALTSGVHTFPAVLQSSGLYSLSSVVTVPSSNFGTQTYTCNVDHKPSNTKVDKTVERKCCVECPPCPAPPVAGPSVFLFPPKPKDTLMISRTPEVTCVVVDVSHEDPEVQFNWYVDGVEVHNAKTKPREEQFNSTFRVVSVLTVVHQDWLNGKEYKCKVSNKGLPAPIEKTISKTKGQPREPQVYTLPPSREEMTKNQVSLTCLVKGFYPSDIAVEWESNGQPENNYKTTPPMLDSDGSFFLYSKLTVDKSRWQQGNVFSCSVMHEALHNHYTQKSLSLSPGK

SEQ ID NO: 8 - protein, 235 aa, Homo sapiens
METPAQLLFLLLLWLPDTTGEIVLTQSPGTLSLSPGERATLSCRASQSVRGRYLAWYQQKPGQAPRLLIYGASSRATGIPDRFSGSGSGTDFTLTISRLEPEDFAVFYCQQYGSSPRTFGQGTKVEIKRTVAAPSVFIFPPSDEQLKSGTASVVCLLNNFYPREAKVQWKVDNALQSGNSQESVTEQDSKDSTYSLSSTLTLSKADYEKHKVYACEVTHQGLSSPVTKSFNRGEC

SEQ ID NO: 9 - protein, 467 aa, Homo sapiens
MEFGLSWLFLVAILKGVQCEVQLLESGGGLVQPGGSLRLSCAASGFTFSSYAMSWVRQAPGKGLEWVSGITGSGGSTYYADSVKGRFTISRDNSKNTLYLQMNSLRAEDTAVYYCAKDPGTTVIMSWFDPWGQGTLVTVSSASTKGPSVFPLAPCSRSTSESTAALGCLVKDYFPEPVTVSWNSGALTSGVHTFPAVLQSSGLYSLSSVVTVPSSNFGTQTYTCNVDHKPSNTKVDKTVERKCCVECPPCPAPPVAGPSVFLFPPKPKDTLMISRTPEVTCVVVDVSHEDPEVQFNWYVDGVEVHNAKTKPREEQFNSTFRVVSVLTVVHQDWLNGKEYKCKVSNKGLPAPIEKTISKTKGQPREPQVYTLPPSREEMTKNQVSLTCLVKGFYPSDIAVEWESNGQPENNYKTTPPMLDSDGSFFLYSKLTVDKSRWQQGNVFSCSVMHEALHNHYTQKSLSLSPGK

SEQ ID NO: 10 - protein, 242 aa, Homo sapiens
MDMRVPAQLLGLLLLWLRGARCDIVMTQTPLSLPVTPGEPASISCRSSQSLLNSVDGSTNLDWYLQKPGQSPQLLIYTLSYRASGVPDRFSGSGSGTDFTLKISRVEAEDVGVYYCMQRIEFPLTFGGGTKVEIKRTVAAPSVFIFPPSDEQLKSGTASVVCLLNNFYPREAKVQWKVDNALQSGNSQESVTEQDSKDSTYSLSSTLTLSKADYEKHKVYACEVTHQGLSSPVTKSFNRGEC

SEQ ID NO: 11 - protein, 465 aa, Homo sapiens
MELGLCWVFLVAILEGVQCEVQLVESGGGLVQPGGSLRLSCAASGFTFSSYSMNWVRQAPGKGLEWVSYISSSGSSIYYADSVKGRFTISRDNAKNSLYLQMNSLRDEDTAVYYCARERYYGDTPFDYWGQGTLVTVSSASTKGPSVFPLAPCSRSTSESTAALGCLVKDYFPEPVTVSWNSGALTSGVHTFPAVLQSSGLYSLSSVVTVPSSNFGTQTYTCNVDHKPSNTKVDKTVERKCCVECPPCPAPPVAGPSVFLFPPKPKDTLMISRTPEVTCVVVDVSHEDPEVQFNWYVDGVEVHNAKTKPREEQFNSTFRVVSVLTVVHQDWLNGKEYKCKVSNKGLPAPIEKTISKTKGQPREPQVYTLPPSREEMTKNQVSLTCLVKGFYPSDIAVEWESNGQPENNYKTTPPMLDSDGSFFLYSKLTVDKSRWQQGNVFSCSVMHEALHNHYTQKSLSLSPGK

SEQ ID NO: 12 - protein, 233 aa, Homo sapiens
MSPSQLIGFLLLWVPASRGEIVLTQSPDFQSVTPKEKVTITCRASQSIGSSLHWYQQKPDQSPKLLIKYASQSFSGVPSRFSGSGSGTDFTLTINSLEAEDAAAYYCHQSSSLPLTFGGGTKVEIKRTVAAPSVFIFPPSDEQLKSGTASVVCLLNNFYPREAKVQWKVDNALQSGNSQESVTEQDSKDSTYSLSSTLTLSKADYEKHKVYACEVTHQGLSSPVTKSFNRGEC

SEQ ID NO: 13 - protein, 463 aa, Homo sapiens
MGSTAILALLLAVLQGVCAEVQLMQSGAEVKKPGESLKISCKGSGYSFSFHWIAWVRQMPGKGLEWMGIIHPGASDTRYSPSFQGQVTISADNSNSATYLQWSSLKASDTAMYFCARQRELDYFDYWGQGTLVTVSSASTKGPSVFPLAPCSRSTSESTAALGCLVKDYFPEPVTVSWNSGALTSGVHTFPAVLQSSGLYSLSSVVTVPSSNFGTQTYTCNVDHKPSNTKVDKTVERKCCVECPPCPAPPVAGPSVFLFPPKPKDTLMISRTPEVTCVVVDVSHEDPEVQFNWYVDGVEVHNAKTKPREEQFNSTFRVVSVLTVVHQDWLNGKEYKCKVSNKGLPAPIEKTISKTKGQPREPQVYTLPPSREEMTKNQVSLTCLVKGFYPSDIAVEWESNGQPENNYKTTPPMLDSDGSFFLYSKLTVDKSRWQQGNVFSCSVMHEALHNHYTQKSLSLSPGK

SEQ ID NO: 14 - protein, 236 aa, Homo sapiens
MDMRVPAQLLGLLLLWLRGARCDIQMTQSPSSLSASVGDRVTITCKASQDINKYVAWYQQKPGKAPKLLIYYTSWLQPGVPSRFSGSGSGTDFTFTISSLQPEDIATYYCLQYDNLLYTFGQGTKLEIKRTVAAPSVFIFPPSDEQLKSGTASVVCLLNNFYPREAKVQWKVDNALQSGNSQESVTEQDSKDSTYSLSSTLTLSKADYEKHKVYACEVTHQGLSSPVTKSFNRGEC

SEQ ID NO: 15 - protein, 467 aa, Homo sapiens
MDMRVPAQLLGLLLLWLRGARCEVQLVESGGGLVQPGGSLRLSCAASGFTFSRYWMNWVRQAPGKGLEWVAQIRLKSDNYATHYAESVKGRFTISRDNAKNSLYLQMNSLRAEDTAVYYCTEGLDYWGQGTTVTVSSASTKGPSVFPLAPSSKSTSGGTAALGCLVKDYFPEPVTVSWNSGALTSGVHTFPAVLQSSGLYSLSSVVTVPSSSLGTQTYICNVNHKPSNTKVDKKVEPKSCDKTHTCPPCPAPELLGGPSVFLFPPKPKDTLMISRTPEVTCVVVDVSHEDPEVKFNWYVDGVEVHNAKTKPREEQYNSTYRVVSVLTVLHQDWLNGKEYKCKVSNKALPAPIEKTISKAKGQPREPQVYTLPPSREEMTKNQVSLTCLVKGFYPSDIAVEWESNGQPENNYKTTPPVLDSDGSFFLYSKLTVDKSRWQQGNVFSCSVMHEALHNHYTQKSLSLSPGK

SEQ ID NO: 16 - protein, 236 aa, Homo sapiens
MDMRVLAQLLGLLLLCFPGARCDIQMTQSPSSLSASVGDRVTITCRASQGISNWLAWYQQKPEKAPKSLIYAASSLQSGVPSRFSGSGSGTDFTLTISSLQPEDFATYYCQQYDSYPRTFGQGTKVEIKRTVAAPSVFIFPPSDEQLKSGTASVVCLLNNFYPREAKVQWKVDNALQSGNSQESVTEQDSKDSTYSLSSTLTLSKADYEKHKVYACEVTHQGLSSPVTKSFNRGEC

SEQ ID NO: 17 - protein, 466 aa, Homo sapiens
MELGLNWVFLVAILEGVHCEVQLVESGGGLVQPGGSLRLSCAASGFTFSSYWMSWVRQAPGKGLEWVAYIKQDGNEKYYVDSVKGRFTISRDNAKNSLYLQMNSLRAEDTAVYYCAREGILWFGDLPTFWGQGTLVTVSSASTKGPSVFPLAPCSRSTSESTAALGCLVKDYFPEPVTVSWNSGALTSGVHTFPAVLQSSGLYSLSSVVTVPSSNFGTQTYTCNVDHKPSNTKVDKTVERKCCVECPPCPAPPVAGPSVFLFPPKPKDTLMISRTPEVTCVVVDVSHEDPEVQFNWYVDGVEVHNAKTKPREEQFNSTFRVVSVLTVVHQDWLNGKEYKCKVSNKGLPAPIEKTISKTKGQPREPQVYTLPPSREEMTKNQVSLTCLVKGFYPSDIAVEWESNGQPENNYKTTPPMLDSDGSFFLYSKLTVDKSRWQQGNVFSCSVMHEALHNHYTQKSLSLSPGK

SEQ ID NO: 18 - protein, 241 aa, Homo sapiens
MDMRLPAQLLGLLMLWVPGSSGDVLMTQSPLSLPVTLGQPASISCRSSQSIVHSNGNTYLEWYLQRPGQSPKLLIYKVSNRFSGVPDRFSGSGSGTDFTLKISRVEAEDVGVYYCFQGSHVPLTFGAGTKLEIKRTVAAPSVFIFPPSDEQLKSGTASVVCLLNNFYPREAKVQWKVDNALQSGNSQESVTEQDSKDSTYSLSSTLTLSKADYEKHKVYACEVTHQGLSSPVTKSFNRGEC

SEQ ID NO: 19 - protein, 470 aa, Homo sapiens
MDTLCSTLLLLTIPSWVLSQVTLKESGPALVKPTQTLTLTCTFSGFSLRTSGMGVGWIRQPPGKALEWLAHIWWDDDKSYNPSLKSQLTISKDTSKNQVVLTMTNMDPVDTATYYCARRNYYYDDYFAYWGQGTLVTVSSASTKGPSVFPLAPSSKSTSGGTAALGCLVKDYFPEPVTVSWNSGALTSGVHTFPAVLQSSGLYSLSSVVTVPSSSLGTQTYICNVNHKPSNTKVDKKVEPKSCDKTHTCPPCPAPELLGGPSVFLFPPKPKDTLMISRTPEVTCVVVDVSHEDPEVKFNWYVDGVEVHNAKTKPREEQYNSTYRVVSVLTVLHQDWLNGKEYKCKVSNKALPAPIEKTISKAKGQPREPQVYTLPPSRDELTKNQVSLTCLVKGFYPSDIAVEWESNGQPENNYKTTPPVLDSDGSFFLYSKLTVDKSRWQQGNVFSCSVMHEALHNHYTQKSLSLSPGK

SEQ ID NO: 20 - protein, 235 aa, Homo sapiens
METPAQLLFLLLLWLPDTTGEIVLTQSPGTLSLSPGERATLSCRASQSVSSSYFAWYQQKPGQAPRLLIYGTSSRATGIPDRFSGSGSGTDFTLTVSRLEPEDFAVYYCQQYDRSPRTFGQGTKVEIKRTVAAPSVFIFPPSDEQLKSGTASVVCLLNNFYPREAKVQWKVDNALQSGNSQESVTEQDSKDSTYSLSSTLTLSKADYEKHKVYACEVTHQGLSSPVTKSFNRGEC

SEQ ID NO: 21 - protein, 463 aa, Homo sapiens
MDWTWRILFLVAAATGAHSQVQLVQSGAAVKKPGASVKVSCKASGYTFTGYYIHWVRQAPGQGLEWMGWINPNSGGTNYAQKFQGRVTMTRDTSISTASMELSRLRSDDTAVYFCARDRWLDAFDIWGQGTMVTVSSASTKGPSVFPLAPCSRSTSESTAALGCLVKDYFPEPVTVSWNSGALTSGVHTFPAVLQSSGLYSLSSVVTVPSSNFGTQTYTCNVDHKPSNTKVDKTVERKCCVECPPCPAPPVAGPSVFLFPPKPKDTLMISRTPEVTCVVVDVSHEDPEVQFNWYVDGVEVHNAKTKPREEQFNSTFRVVSVLTVVHQDWLNGKEYKCKVSNKGLPAPIEKTISKTKGQPREPQVYTLPPSREEMTKNQVSLTCLVKGFYPSDIAVEWESNGQPENNYKTTPPMLDSDGSFFLYSKLTVDKSRWQQGNVFSCSVMHEALHNHYTQKSLSLSPGK

SEQ ID NO: 22 - protein, 235 aa, Homo sapiens
METPAQLLFLLLLWLPDTTGEIVLTQSPGTLSLSPGERATLSCRASQSVSSGYLTWYQQKPGQAPRLLIYGASSRATGIPDRFSGSGSGTDFTLTISRLEPEDFAVYYCQQYGNSLSRFGQGTKLEIKRTVAAPSVFIFPPSDEQLKSGTASVVCLLNNFYPREAKVQWKVDNALQSGNSQESVTEQDSKDSTYSLSSTLTLSKADYEKHKVYACEVTHQGLSSPVTKSFNRGEC

SEQ ID NO: 23 - protein, 474 aa, Homo sapiens
MDMRVPAQLLGLLLLWLRGARCQVQLVESGGGVVQPGRSLRLSCAASGFTFSSYGMHWVRQAPGKGLEWVAVIWYDGSNKYYADSVKGRFIISRDKSKNTLYLQMNSLRAEDTAVYYCARAGGIAAAGLYYYYGMDVWGQGTTVTVSSASTKGPSVFPLAPCSRSTSESTAALGCLVKDYFPEPVTVSWNSGALTSGVHTFPAVLQSSGLYSLSSVVTVPSSNFGTQTYTCNVDHKPSNTKVDKTVERKCCVECPPCPAPPVAGPSVFLFPPKPKDTLMISRTPEVTCVVVDVSHEDPEVQFNWYVDGVEVHNAKTKPREEQFNSTFRVVSVLTVVHQDWLNGKEYKCKVSNKGLPAPIEKTISKTKGQPREPQVYTLPPSREEMTKNQVSLTCLVKGFYPSDIAVEWESNGQPENNYKTTPPMLDSDGSFFLYSKLTVDKSRWQQGNVFSCSVMHEALHNHYTQKSLSLSPGK

SEQ ID NO: 24 - protein, 236 aa, Homo sapiens
MDMRVPAQLLGLLLLWLRGARCSSELTQDPTVSVALGQTVKITCQGDSLRSFYASWYQQKPGQAPVLVFYGKNNRPSGIPDRFSGSSSGNTASLTITGAQAEDEADYYCNSRDSSVYHLVLGGGTKLTVLGQPKANPTVTLFPPSSEELQANKATLVCLISDFYPGAVTVAWKADGSPVKAGVETTKPSKQSNNKYAASSYLSLTPEQWKSHRSYSCQVTHEGSTVEKTVAPTECS

SEQ ID NO: 25 - protein, 478 aa, Homo sapiens
MDMRVPAQLLGLLLLWLRGARCQVQLVQSGAEVKKPGASVKVSCKASGYTFTGYYMHWVRQAPGQGLEWMGWINPNSGGTNYAQKFQGRVTMTRDTSISTAYMELSRLRSDDTAVYFCARDQMSIIMLRGVFPPYYYGMDVWGQGTTVTVSSASTKGPSVFPLAPCSRSTSESTAALGCLVKDYFPEPVTVSWNSGALTSGVHTFPAVLQSSGLYSLSSVVTVPSSNFGTQTYTCNVDHKPSNTKVDKTVERKCCVECPPCPAPPVAGPSVFLFPPKPKDTLMISRTPEVTCVVVDVSHEDPEVQFNWYVDGVEVHNAKTKPREEQFNSTFRVVSVLTVVHQDWLNGKEYKCKVSNKGLPAPIEKTISKTKGQPREPQVYTLPPSREEMTKNQVSLTCLVKGFYPSDIAVEWESNGQPENNYKTTPPMLDSDGSFFLYSKLTVDKSRWQQGNVFSCSVMHEALHNHYTQKSLSLSPGK

SEQ ID NO: 26 - protein, 241 aa, Homo sapiens
MDMRVPAQLLGLLLLWLRGARCDIVMTQSPLSLPVTPGEPASISCRSSQSLLHSNGYNYLDWYLQKPGQSPQLLIYLGSNRASGVPDRFSGSGSGTDFTLKISRVEAEDVGVYYCMQALQTPLTFGGGTKVEIKRTVAAPSVFIFPPSDEQLKSGTASVVCLLNNFYPREAKVQWKVDNALQSGNSQESVTEQDSKDSTYSLSSTLTLSKADYEKHKVYACEVTHQGLSSPVTKSFNRGEC

SEQ ID NO: 27 - protein, 475 aa, Homo sapiens
MDMRVPAQLLGLLLLWLRGARCEVQLVESGGGLVQPGGSLRLSCAASGFTFSSYWMSWVRQAPGKGLEWVASIKQDGSEKYYVDSVKGRFTISRDNARNSLYLQMNSLRAEDTAVYYCARDLVLMVYDIDYYYYGMDVWGQGTTVTVSSASTKGPSVFPLAPCSRSTSESTAALGCLVKDYFPEPVTVSWNSGALTSGVHTFPAVLQSSGLYSLSSVVTVPSSNFGTQTYTCNVDHKPSNTKVDKTVERKCCVECPPCPAPPVAGPSVFLFPPKPKDTLMISRTPEVTCVVVDVSHEDPEVQFNWYVDGVEVHNAKTKPREEQFNSTFRVVSVLTVVHQDWLNGKEYKCKVSNKGLPAPIEKTISKTKGQPREPQVYTLPPSREEMTKNQVSLTCLVKGFYPSDIAVEWESNGQPENNYKTTPPMLDSDGSFFLYSKLTVDKSRWQQGNVFSCSVMHEALHNHYTQKSLSLSPGK

SEQ ID NO: 28 - protein, 241 aa, Homo sapiens
MDMRVPAQLLGLLLLWLRGARCDIVMTQSPLSLPVTPGEPASISCRSSQSLLHSNGYNYLDWYLQKPGQSPQLLIYLGSNRASGVPDRFSGSGSGTHLTLKISRVEAEDVGVYYCMQTLQTPLTFGGGTKVEIKRTVAAPSVFIFPPSDEQLKSGTASVVCLLNNFYPREAKVQWKVDNALQSGNSQESVTEQDSKDSTYSLSSTLTLSKADYEKHKVYACEVTHQGLSSPVTKSFNRGEC

SEQ ID NO: 29 - protein, 475 aa, Homo sapiens
MDMRVPAQLLGLLLLWLRGARCEVQLVESGGGLVQPGGSLRLSCAASGFTFSNYWMSWVRQAPGKGLEWVASIKQDGSEKYYVDSVKGRFAISRDNAKNSLFLQMNSLRAEDTAVYYCARDLVLMVYDIDYYYYGMDVWGQGTTVTVSSASTKGPSVFPLAPCSRSTSESTAALGCLVKDYFPEPVTVSWNSGALTSGVHTFPAVLQSSGLYSLSSVVTVPSSNFGTQTYTCNVDHKPSNTKVDKTVERKCCVECPPCPAPPVAGPSVFLFPPKPKDTLMISRTPEVTCVVVDVSHEDPEVQFNWYVDGVEVHNAKTKPREEQFNSTFRVVSVLTVVHQDWLNGKEYKCKVSNKGLPAPIEKTISKTKGQPREPQVYTLPPSREEMTKNQVSLTCLVKGFYPSDIAVEWESNGQPENNYKTTPPMLDSDGSFFLYSKLTVDKSRWQQGNVFSCSVMHEALHNHYTQKSLSLSPGK

SEQ ID NO: 30 - protein, 235 aa, Homo sapiens
MTCSPLLLTLLIHCTGSWAQSVLTQPPSVSAAPGQKVTISCSGSSSNIGNNYVSWYQQLPGTAPKLLIYDNNKRPSGIPDRFSGSKSGTSTTLGITGLQTGDEADYYCGTWDSRLSAVVFGGGTKLTVLGQPKANPTVTLFPPSSEELQANKATLVCLISDFYPGAVTVAWKADGSPVKAGVETTKPSKQSNNKYAASSYLSLTPEQWKSHRSYSCQVTHEGSTVEKTVAPTECS

SEQ ID NO: 31 - protein, 475 aa, Homo sapiens
MEFGLSWVFLVALLRGVQCQVQLVESGGGVVQPGRSLRLSCAASGFTFSSFGMHWVRQAPGKGLEWVAVISFDGSIKYSVDSVKGRFTISRDNSKNTLFLQMNSLRAEDTAVYYCARDRLNYYDSSGYYHYKYYGMAVWGQGTTVTVSSASTKGPSVFPLAPCSRSTSESTAALGCLVKDYFPEPVTVSWNSGALTSGVHTFPAVLQSSGLYSLSSVVTVPSSNFGTQTYTCNVDHKPSNTKVDKTVERKCCVECPPCPAPPVAGPSVFLFPPKPKDTLMISRTPEVTCVVVDVSHEDPEVQFNWYVDGVEVHNAKTKPREEQFNSTFRVVSVLTVVHQDWLNGKEYKCKVSNKGLPAPIEKTISKTKGQPREPQVYTLPPSREEMTKNQVSLTCLVKGFYPSDIAVEWESNGQPENNYKTTPPMLDSDGSFFLYSKLTVDKSRWQQGNVFSCSVMHEALHNHYTQKSLSLSPGK

SEQ ID NO: 32 - protein, 234 aa, Homo sapiens
MDMRVPAQLLGLLLLWLRGARCYELTQPPSVSVSPGQTATITCSGDKLGERYASWYQQRPGQSPVLVIYQDIKRPSGIPERFSGSNSGNTATLTISGTQAMDEADYFCQAWYSSTNVLFGGGTKLTVLGQPKAAPSVTLFPPSSEELQANKATLVCLISDFYPGAVTVAWKADSSPVKAGVETTTPSKQSNNKYAASSYLSLTPEQWKSHRSYSCQVTHEGSTVEKTVAPTECS

SEQ ID NO: 33 - protein, 466 aa, Homo sapiens
MEFGLSWVFLVALLRGVQCQVQLVESGGGVVQPGRSLRLSCAASGFTFSSYGMHWVRQAPGKGLEWVAVIWYAESNKYYADSVKGRFTISRDNSKNTLYLQMNSLRAEDTAVYYCARAQEGIAPDAFDIWGQGTMVTVSSASTKGPSVFPLAPCSRSTSESTAALGCLVKDYFPEPVTVSWNSGALTSGVHTFPAVLQSSGLYSLSSVVTVPSSNFGTQTYTCNVDHKPSNTKVDKTVERKCCVECPPCPAPPVAGPSVFLFPPKPKDTLMISRTPEVTCVVVDVSHEDPEVQFNWYVDGVEVHNAKTKPREEQFNSTFRVVSVLTVVHQDWLNGKEYKCKVSNKGLPAPIEKTISKTKGQPREPQVYTLPPSREEMTKNQVSLTCLVKGFYPSDIAVEWESNGQPENNYKTTPPMLDSDGSFFLYSKLTVDKSRWQQGNVFSCSVMHEALHNHYTQKSLSLSPGK

SEQ ID NO: 34 - protein, 234 aa, Homo sapiens
MGSTAILGLLLAVLQGGRAEIVLTQSPGTLSLSPGERATLSCRASQSVSSSYLAWHQQKPGQAPRLLIYGASSRATGIPDRFSGSGSGTDFTLTISRLEPEDFAVYYCQQYGSSPWTFGQGTKVEIKRTVAAPSVFIFPPSDEQLKSGTASVVCLLNNFYPREAKVQWKVDNALQSGNSQESVTEQDSKDSTYSLSSTLTLSKADYEKHKVYACEVTHQGLSSPVTKSFNRGEC

SEQ ID NO: 35 - protein, 463 aa, Homo sapiens
MGSTAILGLLLAVLQGGRAEVQLLESGGGLVQPGGSLRLSCAASGFTFSTYVMSWVRQAPGKGLEWVSSISGSGLGSYYADSVKGRFTISRDNSKNTLYLQMNSLRAEDTAVYYCAKEAHRGPFDYWGQGTLVTVSSASTKGPSVFPLAPCSRSTSESTAALGCLVKDYFPEPVTVSWNSGALTSGVHTFPAVLQSSGLYSLSSVVTVPSSNFGTQTYTCNVDHKPSNTKVDKTVERKCCVECPPCPAPPVAGPSVFLFPPKPKDTLMISRTPEVTCVVVDVSHEDPEVQFNWYVDGVEVHNAKTKPREEQFNSTFRVVSVLTVVHQDWLNGKEYKCKVSNKGLPAPIEKTISKTKGQPREPQVYTLPPSREEMTKNQVSLTCLVKGFYPSDIAVEWESNGQPENNYKTTPPMLDSDGSFFLYSKLTVDKSRWQQGNVFSCSVMHEALHNHYTQKSLSLSPGK

SEQ ID NO: 36 - protein, 239 aa, Homo sapiens
MRLLAQLLGLLMLWVPGSSGDIVMTQTPLSSPVTLGQPASISCRSSQSLVHSDGNTYLSWLQQRPGQPPRLLIYKKFNRFSGVPDRFSGSGAGTDFTLKISRVEAEDVGVYYCMQATQIPLTFGPGTKVDIKRTVAAPSVFIFPPSDEQLKSGTASVVCLLNNFYPREAKVQWKVDNALQSGNSQESVTEQDSKDSTYSLSSTLTLSKADYEKHKVYACEVTHQGLSSPVTKSFNRGEC

SEQ ID NO: 37 - protein, 472 aa, Homo sapiens
MEFGLSWVFLVALLRGVQCQVQLVESGGGVVQPGRSLRLSCAASGFTFSFYGMHWVRQAPGKGLEWVAVIWYDGSNKYYADSVKGRFTISRDNSKNTLYLQMNSLRAEDTAVYYCARGGYDYVWGSYRRNSDFDYWGQGTLVTVSSASTKGPSVFPLAPCSRSTSESTAALGCLVKDYFPEPVTVSWNSGALTSGVHTFPAVLQSSGLYSLSSVVTVPSSNFGTQTYTCNVDHKPSNTKVDKTVERKCCVECPPCPAPPVAGPSVFLFPPKPKDTLMISRTPEVTCVVVDVSHEDPEVQFNWYVDGVEVHNAKTKPREEQFNSTFRVVSVLTVVHQDWLNGKEYKCKVSNKGLPAPIEKTISKTKGQPREPQVYTLPPSREEMTKNQVSLTCLVKGFYPSDIAVEWESNGQPENNYKTTPPMLDSDGSFFLYSKLTVDKSRWQQGNVFSCSVMHEALHNHYTQKSLSLSPGK

SEQ ID NO: 38 - protein, 235 aa, Homo sapiens
MEAPAQLLFLLLLWLPDTTGEIVMTQSPATLSVSPGERATLSCRASQSVDSNLAWYRQKPGQAPRLLIYGASTRATGIPARFSGSGSGTEFTLTISSLQSEDFAVYYCQQYINWPPITFGQGTRLEIKRTVAAPSVFIFPPSDEQLKSGTASVVCLLNNFYPREAKVQWKVDNALQSGNSQESVTEQDSKDSTYSLSSTLTLSKADYEKHKVYACEVTHQGLSSPVTKSFNRGEC

SEQ ID NO: 39 - protein, 465 aa, Homo sapiens
MKHLWFFLLLVAAPRWVLSQVQLQESGPGLVKPSETLSLTCTVSGGSISIYYWSWIRQPPGKGLEWIGYVYYSGSTNYNPSLKSRVTISVDTSKNQFSLKLNSVTAADTAVYYCARGGYDFWSGYFDYWGQGTLVTVSSASTKGPSVFPLAPCSRSTSESTAALGCLVKDYFPEPVTVSWNSGALTSGVHTFPAVLQSSGLYSLSSVVTVPSSNFGTQTYTCNVDHKPSNTKVDKTVERKCCVECPPCPAPPVAGPSVFLFPPKPKDTLMISRTPEVTCVVVDVSHEDPEVQFNWYVDGVEVHNAKTKPREEQFNSTFRVVSVLTVVHQDWLNGKEYKCKVSNKGLPAPIEKTISKTKGQPREPQVYTLPPSREEMTKNQVSLTCLVKGFYPSDIAVEWESNGQPENNYKTTPPMLDSDGSFFLYSKLTVDKSRWQQGNVFSCSVMHEALHNHYTQKSLSLSPGK

SEQ ID NO: 40 - protein, 240 aa, Homo sapiens
MVLQTQVFISLLLWISGAYGDIVLTQSPDSLAVSLGERATINCKSSQSILYSSSNENFLTWYQQKPGQPPKLLIYWASTRESGVPDRFSGSGSGTDFTLTISSLQPEDVAVYYCQQYFSVFRTFGQGTRVEIKRTVAAPSVFIFPPSDEQLKSGTASVVCLLNNFYPREAKVQWKVDNALQSGNSQESVTEQDSKDSTYSLSSTLTLSKADYEKHKVYACEVTHQGLSSPVTKSFNRGEC

SEQ ID NO: 41 - protein, 465 aa, Homo sapiens
MDWTWRILFLVAAATGAHSQVQLVQSGAEVKKPGASVKVSCKASGYTFTGYYIHWVRQAPGQGLEWMGWINPNSGGTNSAQKFRGRVTMTRDTSISTAYMELSRLRSDDTAVYYCAREGGYSYGYFDYWGQGTLVTVSSASTKGPSVFPLAPCSRSTSESTAALGCLVKDYFPEPVTVSWNSGALTSGVHTFPAVLQSSGLYSLSSVVTVPSSNFGTQTYTCNVDHKPSNTKVDKTVERKCCVECPPCPAPPVAGPSVFLFPPKPKDTLMISRTPEVTCVVVDVSHEDPEVQFNWYVDGVEVHNAKTKPREEQFNSTFRVVSVLTVVHQDWLNGKEYKCKVSNKGLPAPIEKTISKTKGQPREPQVYTLPPSREEMTKNQVSLTCLVKGFYPSDIAVEWESNGQPENNYKTTPPMLDSDGSFFLYSKLTVDKSRWQQGNVFSCSVMHEALHNHYTQKSLSLSPGK

SEQ ID NO: 42 - protein, 236 aa, Homo sapiens
MDMRVPAQLLGLLLLWFPGARCDIQMTQSPSSLSASVGDRVTITCRASQGIRNDLGWYQQKPGKAPKRLIYAASSLQSGVPSRFSGSGSGTEFTLTISSVQPEDFVTYYCLQHNSNPLTFGGGTKVEIKRTVAAPSVFIFPPSDEQLKSGTASVVCLLNNFYPREAKVQWKVDNALQSGNSQESVTEQDSKDSTYSLSSTLTLSKADYEKHKVYACEVTHQGLSSPVTKSFNRGEC

SEQ ID NO: 43 - protein, 473 aa, Homo sapiens
MEFGLSWVFLVALLRGVQCQVQLVESGGGVVQPGRSLRLSCAASGFTFSSYGMHWVRQAPGKGLEWVAVMWYDGSNKDYVDSVKGRFTISRDNSKNTLYLQMNRLRAEDTAVYYCAREKDHYDILTGYNYYYGLDVWGQGTTVTVSSASTKGPSVFPLAPCSRSTSESTAALGCLVKDYFPEPVTVSWNSGALTSGVHTFPAVLQSSGLYSLSSVVTVPSSNFGTQTYTCNVDHKPSNTKVDKTVERKCCVECPPCPAPPVAGPSVFLFPPKPKDTLMISRTPEVTCVVVDVSHEDPEVQFNWYVDGVEVHNAKTKPREEQFNSTFRVVSVLTVVHQDWLNGKEYKCKVSNKGLPAPIEKTISKTKGQPREPQVYTLPPSREEMTKNQVSLTCLVKGFYPSDIAVEWESNGQPENNYKTTPPMLDSDGSFFLYSKLTVDKSRWQQGNVFSCSVMHEALHNHYTQKSLSLSPGK

SEQ ID NO: 44 - protein, 235 aa, Homo sapiens
METPAQLLFLLLLWLPDTTGEIVLTQSPGTLSLSPGERATLSCRASQYISNTYLAWFQQKPGQAPRLLIYGAATRATGIPDRFSGSGSGTDFTFTISRLEPEDFAVYYCQQYGSSPWTFGQGTTVEIKRTVAAPSVFIFPPSDEQLKSGTASVVCLLNNFYPREAKVQWKVDNALQSGNSQESVTEQDSKDSTYSLSSTLTLSKADYEKHKVYACEVTHQGLSSPVTKSFNRGEC

SEQ ID NO: 45 - protein, 463 aa, Homo sapiens
MDWTWRILFLVAAATGAHSQVQLVQSGAEVKKPGASVKVSCKASGYTFTGYYMHWVRQAPGQGLEWMGWINPNSGGTNYAQRFRGRVTMTRDTSISTAYMELSRLRSDDTAVYYCARAPYDWTFDYWGQGTLVTVSSASTKGPSVFPLAPCSRSTSESTAALGCLVKDYFPEPVTVSWNSGALTSGVHTFPAVLQSSGLYSLSSVVTVPSSNFGTQTYTCNVDHKPSNTKVDKTVERKCCVECPPCPAPPVAGPSVFLFPPKPKDTLMISRTPEVTCVVVDVSHEDPEVQFNWYVDGVEVHNAKTKPREEQFNSTFRVVSVLTVVHQDWLNGKEYKCKVSNKGLPAPIEKTISKTKGQPREPQVYTLPPSREEMTKNQVSLTCLVKGFYPSDIAVEWESNGQPENNYKTTPPMLDSDGSFFLYSKLTVDKSRWQQGNVFSCSVMHEALHNHYTQKSLSLSPGK

SEQ ID NO: 46 - protein, 236 aa, Homo sapiens
MDMRVPAQLLGLLLLWLRGARCDIQMTQSPSSVSASVGDRVTITCRASQGISNWLAWYQQKPGTAPKLLIYAASSLQSGVPSRFSGSGSGTDFTLTISSLQPEDFATYYCQQANSFPFTFGPGTKVDIKRTVAAPSVFIFPPSDEQLKSGTASVVCLLNNFYPREAKVQWKVDNALQSGNSQESVTEQDSKDSTYSLSSTLTLSKADYEKHKVYACEVTHQGLSSPVTKSFNRGEC

SEQ ID NO: 47 - protein, 469 aa, Homo sapiens
MDMRVPAQLLGLLLLWLRGARCQVQLVQSGTEVKKPGASMKVSCKASGYTFTSYYMHWVRQAPGQGLEWMGIINPSGDSTSYAQKFQGRVTMTRDTSTNTVYMELSSLRSEDTAMYYCARDVEVRGISHFDYWGQGTLVTVSSASTKGPSVFPLAPCSRSTSESTAALGCLVKDYFPEPVTVSWNSGALTSGVHTFPAVLQSSGLYSLSSVVTVPSSNFGTQTYTCNVDHKPSNTKVDKTVERKCCVECPPCPAPPVAGPSVFLFPPKPKDTLMISRTPEVTCVVVDVSHEDPEVQFNWYVDGVEVHNAKTKPREEQFNSTFRVVSVLTVVHQDWLNGKEYKCKVSNKGLPAPIEKTISKTKGQPREPQVYTLPPSREEMTKNQVSLTCLVKGFYPSDIAVEWESNGQPENNYKTTPPMLDSDGSFFLYSKLTVDKSRWQQGNVFSCSVMHEALHNHYTQKSLSLSPGK

SEQ ID NO: 48 - protein, 238 aa, Homo sapiens
MGWSCIILFLVATATGVHSDIQLTQSPSSLSASVGDRVTMSCKSSQSVLYSANHKNYLAWYQQKPGKAPKLLIYWASTRESGVPSRFSGSGSGTDFTFTISSLQPEDIATYYCHQYLSSWTFGGGTKVQIKRTVAAPSVFIFPPSDEQLKSGTASVVCLLNNFYPREAKVQWKVDNALQSGNSQESVTEQDSKDSTYSLSSTLTLSKADYEKHKVYACEVTHQGLSSPVTKSFNRGEC

SEQ ID NO: 49 - protein, 465 aa, Homo sapiens
MGWSCIILFLVATATGVHSQVQLVQSGAEVKKPGSSVKVSCKASGYTFTSYWLHWVRQAPGQGLEWIGYINPRNDYTEYNQNFKDKATITADESTNTAYMELSSLRSEDTAFYFCARRDITTFYWGQGTTVTVSSASTKGPSVFPLAPSSKSTSGGTAALGCLVKDYFPEPVTVSWNSGALTSGVHTFPAVLQSSGLYSLSSVVTVPSSSLGTQTYICNVNHKPSNTKVDKRVEPKSCDKTHTCPPCPAPELLGGPSVFLFPPKPKDTLMISRTPEVTCVVVDVSHEDPEVKFNWYVDGVEVHNAKTKPREEQYNSTYRVVSVLTVLHQDWLNGKEYKCKVSNKALPAPIEKTISKAKGQPREPQVYTLPPSREEMTKNQVSLTCLVKGFYPSDIAVEWESNGQPENNYKTTPPVLDSDGSFFLYSKLTVDKSRWQQGNVFSCSVMHEALHNHYTQKSLSLSPGK

SEQ ID NO: 50 - protein, 235 aa, Homo sapiens
METPAQLLFLLLLWLPDTTGEIVLTQSPGTLSLSPGERATLSCRASQSVSSSYLAWYQQKPGQAPRLLIYGASSRATGIPDRFSGSGSGTDFTLTISRLEPEDFAVYYCQRSGGSSFTFGPGTKVDIKRTVAAPSVFIFPPSDEQLKSGTASVVCLLNNFYPREAKVQWKVDNALQSGNSQESVTEQDSKDSTYSLSSTLTLSKADYEKHKVYACEVTHQGLSSPVTKSFNRGEC

SEQ ID NO: 51 - protein, 466 aa, Homo sapiens
MGSTAILALLLAVLQGVCAEVQLVQSGAEVKKPGESLKISCKGSGYNFTSYWIGWVRQMPGKGLELMGIIYPGDSDTRYSPSFQGQVTISADKSISTAYLQWSSLKASDTAMYYCGSGSYFYFDLWGRGTLVTVSSASTKGPSVFPLAPSSKSTSGGTAALGCLVKDYFPEPVTVSWNSGALTSGVHTFPAVLQSSGLYSLSSVVTVPSSSLGTQTYICNVNHKPSNTKVDKKVEPKSCDKTHTCPPCPAPELLGGPSVFLFPPKPKDTLMISRTPEVTCVVVDVSHEDPEVKFNWYVDGVEVHNAKTKPREEQYNSTYRVVSVLTVLHQDWLNGKEYKCKVSNKALPAPIEKTISKAKGQPREPQVYTLPPSRDELTKNQVSLTCLVKGFYPSDIAVEWESNGQPENNYKTTPPVLDSDGSFFLYSKLTVDKSRWQQGNVFSCSVMHEALHNHYTQKSLSLSPGK

SEQ ID NO: 52 - protein, 241 aa, Homo sapiens
MDMRVPAQLLGLLLLWLRGARCDIVMTQSPLSLPVTPGEPASISCRSSQSLLHSHGYNYLDWYLQKPGQSPQLLIYLGSNRASGVPDRFSGSGSGTDFTLKISRVEAEDVGVYYCMQGTHWPPTFGQGTKLEIKRTVAAPSVFIFPPSDEQLKSGTASVVCLLNNFYPREAKVQWKVDNALQSGNSQESVTEQDSKDSTYSLSSTLTLSKADYEKHKVYACEVTHQGLSSPVTKSFNRGEC

SEQ ID NO: 53 - protein, 470 aa, Homo sapiens
MDMRVPAQLLGLLLLWLRGARCEVQLVQSGGGVVQPGRSLRLSCAASGFTFSSYGMHWVRQAPGKGLEWVSYISSSGSTIYYADSVKGRFTISRDNAKNSLYLQMNSLRAEDTAVYYCARDLLDYDLLTGYGYWGQGTLVTVSSASTKGPSVFPLAPCSRSTSESTAALGCLVKDYFPEPVTVSWNSGALTSGVHTFPAVLQSSGLYSLSSVVTVPSSNFGTQTYTCNVDHKPSNTKVDKTVERKCCVECPPCPAPPVAGPSVFLFPPKPKDTLMISRTPEVTCVVVDVSHEDPEVQFNWYVDGVEVHNAKTKPREEQFNSTFRVVSVLTVVHQDWLNGKEYKCKVSNKGLPAPIEKTISKTKGQPREPQVYTLPPSREEMTKNQVSLTCLVKGFYPSDIAVEWESNGQPENNYKTTPPMLDSDGSFFLYSKLTVDKSRWQQGNVFSCSVMHEALHNHYTQKSLSLSPGK

SEQ ID NO: 54 - protein, 235 aa, Homo sapiens
METPAQLLFLLLLWLPDTTGEIVLTQSPGTLSLSPGERATLSCRASQGISRSYLAWYQQKPGQAPSLLIYGASSRATGIPDRFSGSGSGTDFTLTISRLEPEDFAVYYCQQFGSSPWTFGQGTKVEIKRTVAAPSVFIFPPSDEQLKSGTASVVCLLNNFYPREAKVQWKVDNALQSGNSQESVTEQDSKDSTYSLSSTLTLSKADYEKHKVYACEVTHQGLSSPVTKSFNRGEC

SEQ ID NO: 55 - protein, 471 aa, Homo sapiens
MKHLWFFLLLVAAPRWVLSQVQLQESGPGLVKPSQTLSLTCTVSGGSISSGDYFWSWIRQLPGKGLEWIGHIHNSGTTYYNPSLKSRVTISVDTSKKQFSLRLSSVTAADTAVYYCARDRGGDYYYGMDVWGQGTTVTVSSASTKGPSVFPLAPSSKSTSGGTAALGCLVKDYFPEPVTVSWNSGALTSGVHTFPAVLQSSGLYSLSSVVTVPSSSLGTQTYICNVNHKPSNTKVDKRVEPKSCDKTHTCPPCPAPELLGGPSVFLFPPKPKDTLMISRTPEVTCVVVDVSHEDPEVKFNWYVDGVEVHNAKTKPREEQYNSTYRVVSVLTVLHQDWLNGKEYKCKVSNKALPAPIEKTISKAKGQPREPQVYTLPPSREEMTKNQVSLTCLVKGFYPSDIAVEWESNGQPENNYKTTPPVLDSDGSFFLYSKLTVDKSRWQQGNVFSCSVMHEALHNHYTQKSLSLSPGK

SEQ ID NO: 56 - protein, 236 aa, Homo sapiens
MDMRVPAQLLGLLLLWLSGARCDIQMTQSPSSLSASVGDRVTITCQASQDISNYLNWYQQKPGKAPKLLIYDASNLETGVPSRFSGSGSGTDFTFTISSLQPEDIATYFCQHFDHLPLAFGGGTKVEIKRTVAAPSVFIFPPSDEQLKSGTASVVCLLNNFYPREAKVQWKVDNALQSGNSQESVTEQDSKDSTYSLSSTLTLSKADYEKHKVYACEVTHQGLSSPVTKSFNRGEC

SEQ ID NO: 57 - protein, 464 aa, Homo sapiens
MKHLWFFLLLVAAPRWVLSQVQLQESGPGLVKPSETLSLTCTVSGGSVSSGDYYWTWIRQSPGKGLEWIGHIYYSGNTNYNPSLKSRLTISIDTSKTQFSLKLSSVTAADTAIYYCVRDRVTGAFDIWGQGTMVTVSSASTKGPSVFPLAPCSRSTSESTAALGCLVKDYFPEPVTVSWNSGALTSGVHTFPAVLQSSGLYSLSSVVTVPSSNFGTQTYTCNVDHKPSNTKVDKTVERKCCVECPPCPAPPVAGPSVFLFPPKPKDTLMISRTPEVTCVVVDVSHEDPEVQFNWYVDGVEVHNAKTKPREEQFNSTFRVVSVLTVVHQDWLNGKEYKCKVSNKGLPAPIEKTISKTKGQPREPQVYTLPPSREEMTKNQVSLTCLVKGFYPSDIAVEWESNGQPENNYKTTPPMLDSDGSFFLYSKLTVDKSRWQQGNVFSCSVMHEALHNHYTQKSLSLSPGK

SEQ ID NO: 58 - protein, 236 aa, Homo sapiens
METPAQLLFLLLLWLPDTASEIVLTQSPGTLSLSPGERATLSCRASQSVSNSYLAWYQQKPGQAPRLLIYGASSRAPGIPDRFSGSGSGTDFTLTISRLEPEDFAVYYCQQYDHSAGWTFGQGTKVEIKRTVAAPSVFIFPPSDEQLKSGTASVVCLLNNFYPREAKVQWKVDNALQSGNSQESVTEQDSKDSTYSLSSTLTLSKADYEKHKVYACEVTHQGLSSPVTKSFNRGEC

SEQ ID NO: 59 - protein, 460 aa, Homo sapiens
MGSTAILGLLLAVLQGVASEVQLVESGGGLVQPGGSLRLSCAASGFTFSRNAMFWVRQAPGKGLEWVSGIGTGGATSYADSVKGRFTISRDNAKNSLYLQMNSLRAEDTAVYYCARGRYYFPWWGQGTLVTVSSASTKGPSVFPLAPCSRSTSESTAALGCLVKDYFPEPVTVSWNSGALTSGVHTFPAVLQSSGLYSLSSVVTVPSSNFGTQTYTCNVDHKPSNTKVDKTVERKCCVECPPCPAPPVAGPSVFLFPPKPKDTLMISRTPEVTCVVVDVSHEDPEVQFNWYVDGVEVHNAKTKPREEQFNSTFRVVSVLTVVHQDWLNGKEYKCKVSNKGLPAPIEKTISKTKGQPREPQVYTLPPSREEMTKNQVSLTCLVKGFYPSDIAVEWESNGQPENNYKTTPPMLDSDGSFFLYSKLTVDKSRWQQGNVFSCSVMHEALHNHYTQKSLSLSPGK

SEQ ID NO: 60 - protein, 234 aa, Homo sapiens
METPAQLLFLLLLWLPDTTGEIVLTQSPGTLSLSPGERATLSCRASQSVSSSYLAWYQQKPGQAPRLLIYGASRRATGIPDRFSGSGSGTDFTLTISRLEPEDFAVYYCQRYGSSHTFGQGTKLEISRTVAAPSVFIFPPSDEQLKSGTASVVCLLNNFYPREAKVQWKVDNALQSGNSQESVTEQDSKDSTYSLSSTLTLSKADYEKHKVYACEVTHQGLSSPVTKSFNRGEC

SEQ ID NO: 61 - protein, 467 aa, Homo sapiens
MGSTAILALLLAVLQGVCAEVQLVQSGAEVKKPGESLKISCKVSGYFFTTYWIGWVRQMPGKGLEYMGIIYPGDSDTRYSPSFQGQVTISADKSISTAYLQWSSLKASDTAMYYCARGGNWNCFDYWGQGTLVTVSSASTKGPSVFPLAPSSKSTSGGTAALGCLVKDYFPEPVTVSWNSGALTSGVHTFPAVLQSSGLYSLSSVVTVPSSSLGTQTYICNVNHKPSNTKVDKRVEPKSCDKTHTCPPCPAPELLGGPSVFLFPPKPKDTLMISRTPEVTCVVVDVSHEDPEVKFNWYVDGVEVHNAKTKPREEQYNSTYRVVSVLTVLHQDWLNGKEYKCKVSNKALPAPIEKTISKAKGQPREPQVYTLPPSRDELTKNQVSLTCLVKGFYPSDIAVEWESNGQPENNYKTTPPVLDSDGSFFLYSKLTVDKSRWQQGNVFSCSVMHEALHNHYTQKSLSLSPGK

SEQ ID NO: 62 - protein, 241 aa, Homo sapiens
MDMRVPAQLLGLLLLWLRGARCDVVMTQSPLSLPVTPGEPASISCRSSQSLLHSNGYNYLDWYLQKPGQSPQLLIYLGSNRASGVPDRFSGSGSGTDFTLKISRVEAEDVGVYYCMQGTHWPLTFGQGTKVEIKRTVAAPSVFIFPPSDEQLKSGTASVVCLLNNFYPREAKVQWKVDNALQSGNSQESVTEQDSKDSTYSLSSTLTLSKADYEKHKVYACEVTHQGLSSPVTKSFNRGEC

SEQ ID NO: 63 - protein, 471 aa, Homo sapiens
MDMRVPAQLLGLLLLWLRGARCQVQLQESGPGLVKPSGTLSLTCAVSGGSISSSNWWSWVRQPPGKGLEWIGEIYHSGSTNYNPSLKSRVTISVDKSKNQFSLKLSSVTAADTAVYYCARWTGRTDAFDIWGQGTMVTVSSASTKGPSVFPLAPSSKSTSGGTAALGCLVKDYFPEPVTVSWNSGALTSGVHTFPAVLQSSGLYSLSSVVTVPSSSLGTQTYICNVNHKPSNTKVDKKVEPKSCDKTHTCPPCPAPELLGGPSVFLFPPKPKDTLMISRTPEVTCVVVDVSHEDPEVKFNWYVDGVEVHNAKTKPREEQYNSTYRVVSVLTVLHQDWLNGKEYKCKVSNKALPAPIEKTISKAKGQPREPQVYTLPPSRDELTKNQVSLTCLVKGFYPSDIAVEWESNGQPENNYKTTPPVLDSDGSFFLYSKLTVDKSRWQQGNVFSCSVMHEALHNHYTQKSLSLSPGK

SEQ ID NO: 64 - protein, 234 aa, Homo sapiens
MEAPAQLLFLLLLWLPDTTGEIVMTQSPATLSVSPGERATLSCRASQSVSSNLAWFQQKPGQAPRPLIYDASTRATGVPARFSGSGSGTDFTLTISSLQSEDFAVYYCQQYDNWPLTFGGGTKVEIKRTVAAPSVFIFPPSDEQLKSGTASVVCLLNNFYPREAKVQWKVDNALQSGNSQESVTEQDSKDSTYSLSSTLTLSKADYEKHKVYACEVTHQGLSSPVTKSFNRGEC

SEQ ID NO: 65 - protein, 461 aa, Homo sapiens
MEWTWRVLFLVAAATGAHSQVQLVQSGAEVKKPGASVKVSCKASGYTFTRYGISWVRQAPGQGLEWMGWISTYSGNTNYAQKLQGRVTMTTDTSTSTAYMELRSLRSDDTAVYYCARRQLYFDYWGQGTLVTVSSASTKGPSVFPLAPCSRSTSESTAALGCLVKDYFPEPVTVSWNSGALTSGVHTFPAVLQSSGLYSLSSVVTVPSSNFGTQTYTCNVDHKPSNTKVDKTVERKCCVECPPCPAPPVAGPSVFLFPPKPKDTLMISRTPEVTCVVVDVSHEDPEVQFNWYVDGVEVHNAKTKPREEQFNSTFRVVSVLTVVHQDWLNGKEYKCKVSNKGLPAPIEKTISKTKGQPREPQVYTLPPSREEMTKNQVSLTCLVKGFYPSDIAVEWESNGQPENNYKTTPPMLDSDGSFFLYSKLTVDKSRWQQGNVFSCSVMHEALHNHYTQKSLSLSPGK

SEQ ID NO: 66 - protein, 239 aa, Homo sapiens
MRLPAQLLGLLMLWIPGSSADIVMTQTPLSLSVTPGQPASISCKSGQSLLHSDGKTYLYWYLQKPGQPPQFLIYEVSNRFSRVPDRFSGSGSGTDFTLRISRVEAEDVGIYYCMQSIQLPWTFGQGTQVEIKRTVAAPSVFIFPPSDEQLKSGTASVVCLLNNFYPREAKVQWKVDNALQSGNSQESVTEQDSKDSTYSLSSTLTLSKADYEKHKVYACEVTHQGLSSPVTKSFNRGEC

SEQ ID NO: 67 - protein, 459 aa, Homo sapiens
MEFGLSWVFLVALLRGVQCQVQLVESGGGVVQPGRSLRLSCAASGFTFSGYGMHWVRQAPGKGLEWVAVISYDGNDKYYADSVKGRFTISRDNAKNTLYLQMNSLRAEDTAVYYCARELRVLWGQGTLVTVSSASTKGPSVFPLAPCSRSTSESTAALGCLVKDYFPEPVTVSWNSGALTSGVHTFPAVLQSSGLYSLSSVVTVPSSNFGTQTYTCNVDHKPSNTKVDKTVERKCCVECPPCPAPPVAGPSVFLFPPKPKDTLMISRTPEVTCVVVDVSHEDPEVQFNWYVDGVEVHNAKTKPREEQFNSTFRVVSVLTVVHQDWLNGKEYKCKVSNKGLPAPIEKTISKTKGQPREPQVYTLPPSREEMTKNQVSLTCLVKGFYPSDIAVEWESNGQPENNYKTTPPMLDSDGSFFLYSKLTVDKSRWQQGNVFSCSVMHEALHNHYTQKSLSLSPGK

SEQ ID NO: 68 - protein, 235 aa, Homo sapiens
MDMRVPAQLLGLLLLWLRGARCDIQMTQSPSSLSASVGDRVTITCRASQDISSYLNWYQQKPGKAPKLLIYSTSRLNSGVPSRFSGSGSGTDFTLTISSLQPEDFATYYCQQDIKHPTFGQGTKVEIKRTVAAPSVFIFPPSDEQLKSGTASVVCLLNNFYPREAKVQWKVDNALQSGNSQESVTEQDSKDSTYSLSSTLTLSKADYEKHKVYACEVTHQGLSSPVTKSFNRGEC

SEQ ID NO: 69 - protein, 465 aa, Homo sapiens
MDWTWRILFLVAAATGAHSEVQLVQSGAEVKKPGSSVKVSCKASGFTFTDYIMHWVRQAPGQGLEWMGYINPYNDDTEYNEKFKGRVTITADKSTSTAYMELSSLRSEDTAVYYCARSIYYYDAPFAYWGQGTLVTVSSASTKGPSVFPLAPCSRSTSESTAALGCLVKDYFPEPVTVSWNSGALTSGVHTFPAVLQSSGLYSLSSVVTVPSSNFGTQTYTCNVDHKPSNTKVDKTVERKCCVECPPCPAPPVAGPSVFLFPPKPKDTLMISRTPEVTCVVVDVSHEDPEVQFNWYVDGVEVHNAKTKPREEQFNSTFRVVSVLTVVHQDWLNGKEYKCKVSNKGLPAPIEKTISKTKGQPREPQVYTLPPSREEMTKNQVSLTCLVKGFYPSDIAVEWESNGQPENNYKTTPPMLDSDGSFFLYSKLTVDKSRWQQGNVFSCSVMHEALHNHYTQKSLSLSPGK

SEQ ID NO: 70 - protein, 233 aa, Homo sapiens
MGSTAILGLLLAVLQGGRASYVLTQPPSVSVAPGQTARITCGGNNLGSKSVHWYQQKPGQAPVLVVYDDSDRPSWIPERFSGSNSGNTATLTISRGEAGDEADYYCQVWDSSSDHVVFGGGTKLTVLGQPKAAPSVTLFPPSSEELQANKATLVCLISDFYPGAVTVAWKADSSPVKAGVETTTPSKQSNNKYAASSYLSLTPEQWKSHRSYSCQVTHEGSTVEKTVAPTECS

SEQ ID NO: 71 - protein, 467 aa, Homo sapiens
MGSTAILGLLLAVLQGGRAQMQLVESGGGVVQPGRSLRLSCAASGFTFRTYGMHWVRQAPGKGLEWVAVIWYDGSNKHYADSVKGRFTITRDNSKNTLNLQMNSLRAEDTAVYYCARAPQWELVHEAFDIWGQGTMVTVSSASTKGPSVFPLAPCSRSTSESTAALGCLVKDYFPEPVTVSWNSGALTSGVHTFPAVLQSSGLYSLSSVVTVPSSNFGTQTYTCNVDHKPSNTKVDKTVERKCCVECPPCPAPPVAGPSVFLFPPKPKDTLMISRTPEVTCVVVDVSHEDPEVQFNWYVDGVEVHNAKTKPREEQFNSTFRVVSVLTVVHQDWLNGKEYKCKVSNKGLPAPIEKTISKTKGQPREPQVYTLPPSREEMTKNQVSLTCLVKGFYPSDIAVEWESNGQPENNYKTTPPMLDSDGSFFLYSKLTVDKSRWQQGNVFSCSVMHEALHNHYTQKSLSLSPGK

SEQ ID NO: 72 - protein, 234 aa, Homo sapiens
MGVPTHLLGLLLLWITHAICDIRMTQSPASLSASLGETVNIECLASEDIYSDLAWYQQKPGKSPQLLIYNANSLQNGVPSRFSGSGSGTQYSLKINSLQSEDVATYFCQQYNNYPPTFGGGTKLELKRADAAPTVSIFPPSTEQLATGGASVVCLMNNFYPRDISVKWKIDGTERRDGVLDSVTDQDSKDSTYSMSSTLSLTKADYESHNLYTCEVVHKTSSSPVVKSFNRNEC

SEQ ID NO: 73 - protein, 465 aa, Homo sapiens
MDIRLSLAFLVLFIKGVQCEVQLVESGGGLVQPANSLKLSCAASGFTFSDYAMAWVRQSPKKGLEWVATIIYDGSSTYYRDSVKGRFTISRDNAKSTLYLQMDSLRSEDTATYYCATGLGIATDYFDYWGQGVLVTVSSAETTAPSVYPLAPGTALKSNSMVTLGCLVKGYFPEPVTVTWNSGALSSGVHTFPAVLQSGLYTLTSSVTVPSSTWPSQTVTCNVAHPASSTKVDKKIVPRNCGGDCKPCICTGSEVSSVFIFPPKPKDVLTITLTPKVTCVVVDISQDDPEVHFSWFVDDVEVHTAQTRPPEEQFNSTFRSVSELPILHQDWLNGRTFRCKVTSAAFPSPIEKTISKPEGRTQVPHVYTMSPTKEEMTQNEVSITCMVKGFYPPDIYVEWQMNGQPQENYKNTPPTMDTDGSYFLYSKLNVKKEKWQQGNTFTCSVLHEGLHNHHTEKSLSHSPGK

SEQ ID NO: 74 - protein, 237 aa, Homo sapiens
MDMRVPAQLLGLLLLWLRGARCESALTQPASVSGSPGQSITISCTGTSSDVGGYNSVSWYQQHPGKAPKLMIYEVSNRPSGVSNRFSGSKSGNTASLTISGLQAEDEADYYCNSYTSTSMVFGGGTKLTVLGQPKAAPSVTLFPPSSEELQANKATLVCLISDFYPGAVTVAWKADSSPVKAGVETTTPSKQSNNKYAASSYLSLTPEQWKSHRSYSCQVTHEGSTVEKTVAPTECS

SEQ ID NO: 75 - protein, 460 aa, Homo sapiens
MDWTWRILFLVAAATGVHSEVQLVQSGAEVKKPGASVKVSCKASGYTLTSYGISWVRQAPGQGLEWMGWVSFYNGNTNYAQKLQGRGTMTTDPSTSTAYMELRSLRSDDTAVYYCARGYGMDVWGQGTTVTVSSASTKGPSVFPLAPCSRSTSESTAALGCLVKDYFPEPVTVSWNSGALTSGVHTFPAVLQSSGLYSLSSVVTVPSSNFGTQTYTCNVDHKPSNTKVDKTVERKCCVECPPCPAPPVAGPSVFLFPPKPKDTLMISRTPEVTCVVVDVSHEDPEVQFNWYVDGVEVHNAKTKPREEQFNSTFRVVSVLTVVHQDWLNGKEYKCKVSNKGLPAPIEKTISKTKGQPREPQVYTLPPSREEMTKNQVSLTCLVKGFYPSDIAVEWESNGQPENNYKTTPPMLDSDGSFFLYSKLTVDKSRWQQGNVFSCSVMHEALHNHYTQKSLSLSPGK

SEQ ID NO: 76 - protein, 234 aa, Homo sapiens
METPAQLLFLLLLWLPDTTGEIVMTQSPATLSVSPGERATLSCRASQSVSSNLAWYQQKPGQAPRLLIYGAATRATGIPARVSGSGSGTEFTLTISSLQSEDFAVYYCQQYNNWPLTFGGGTKVEIKRTVAAPSVFIFPPSDEQLKSGTASVVCLLNNFYPREAKVQWKVDNALQSGNSQESVTEQDSKDSTYSLSSTLTLSKADYEKHKVYACEVTHQGLSSPVTKSFNRGEC

SEQ ID NO: 77 - protein, 472 aa, Homo sapiens
MDMRVPAQLLGLLLLWLRGARCQVQLVESGGGVVQPGRSLRLSCAASGFTFSNYGMHWVRQAPGEGLEWVAAIWFDASDKYYADAVKGRFTISRDNSKNTLYLQMNSLRAEDTAVYYCARDQAIFGVVPDYWGQGTLVTVSSASTKGPSVFPLAPSSKSTSGGTAALGCLVKDYFPEPVTVSWNSGALTSGVHTFPAVLQSSGLYSLSSVVTVPSSSLGTQTYICNVNHKPSNTKVDKKVEPKSCDKTHTCPPCPAPELLGGPSVFLFPPKPKDTLMISRTPEVTCVVVDVSHEDPEVKFNWYVDGVEVHNAKTKPCEEQYGSTYRCVSVLTVLHQDWLNGKEYKCKVSNKALPAPIEKTISKAKGQPREPQVYTLPPSREEMTKNQVSLTCLVKGFYPSDIAVEWESNGQPENNYKTTPPVLDSDGSFFLYSKLTVDKSRWQQGNVFSCSVMHEALHNHYTQKSLSLSPGK

SEQ ID NO: 78 - protein, 231 aa, Homo sapiens
MAWIPLFLGVLAYCTGSVASYEVTQAPSVSVSPGQTASITCSGDKLGDKYACWYQQKPGQSPVLVIYQDSKRPSGIPERFSGSNSGNTATLTISGTQAMDEADYYCQAWDSSTAVFGGGTKLTVLGQPKAAPSVTLFPPSSEELQANKATLVCLISDFYPGAVTVAWKADSSPVKAGVETTTPSKQSNNKYAASSYLSLTPEQWKSHRSYSCQVTHEGSTVEKTVAPTECS

SEQ ID NO: 79 - protein, 467 aa, Homo sapiens
MDWTWSILFLVAAATGAHSQVQLVQSGAEVKKPGASVKVSCKASGYTFTSYGLSWVRQAPGQGLEWMGWIIPYNGNTNSAQKLQGRVTMTTDTSTSTAYMELRSLRSDDTAVYFCARDRDYGVNYDAFDIWGQGTMVTVSSASTKGPSVFPLAPCSRSTSESTAALGCLVKDYFPEPVTVSWNSGALTSGVHTFPAVLQSSGLYSLSSVVTVPSSNFGTQTYTCNVDHKPSNTKVDKTVERKCCVECPPCPAPPVAGPSVFLFPPKPKDTLMISRTPEVTCVVVDVSHEDPEVQFNWYVDGVEVHNAKTKPREEQFNSTFRVVSVLTVVHQDWLNGKEYKCKVSNKGLPAPIEKTISKTKGQPREPQVYTLPPSREEMTKNQVSLTCLVKGFYPSDIAVEWESNGQPENNYKTTPPMLDSDGSFFLYSKLTVDKSRWQQGNVFSCSVMHEALHNHYTQKSLSLSPGK

SEQ ID NO: 80 - protein, 235 aa, Homo sapiens
MAWAPLLLTLLAHCTGSWANFMLTQPHSVSESPGKTVAISCTRNSGSIASNSVQWYQQRPGSSPTTVIFEDNQRPSGVPDRFSGSIDSSSNSASLTISGLKTEDEADYYCQSYDSNNWVFGGGTKLTVLGQPKANPTVTLFPPSSEELQANKATLVCLISDFYPGAVTVAWKADGSPVKAGVETTKPSKQSNNKYAASSYLSLTPEQWKSHRSYSCQVTHEGSTVEKTVAPTECS

SEQ ID NO: 81 - protein, 470 aa, Homo sapiens
MEFGLSWVFLVALLRGVQCQVQLVESGGGVVQPGRSLRLSCAASGFTFSSYVMHWVRQAPGKGLEWVAVIWYDGSNKYYADSVKGRFTISRDNSKNTLYLQMNSLRAEDTAVYYCAREGYDYGEDYYYYGMDVWGQGTTVTVSSASTKGPSVFPLAPCSRSTSESTAALGCLVKDYFPEPVTVSWNSGALTSGVHTFPAVLQSSGLYSLSSVVTVPSSNFGTQTYTCNVDHKPSNTKVDKTVERKCCVECPPCPAPPVAGPSVFLFPPKPKDTLMISRTPEVTCVVVDVSHEDPEVQFNWYVDGVEVHNAKTKPREEQFNSTFRVVSVLTVVHQDWLNGKEYKCKVSNKGLPAPIEKTISKTKGQPREPQVYTLPPSREEMTKNQVSLTCLVKGFYPSDIAVEWESNGQPENNYKTTPPMLDSDGSFFLYSKLTVDKSRWQQGNVFSCSVMHEALHNHYTQKSLSLSPGK

SEQ ID NO: 82 - protein, 236 aa, Homo sapiens
MDMRVPAQLLGLLLLWLRGARCDIQMTQSPSSLSASVGDRVTITCRASQDISNYLNWYQQKPGKAPKLLIYYTSRLLSGVPSRFSGSGSGTDFTLTISSLQPEDFATYYCQQGDTLPYTFGGGTKVEIKRTVAAPSVFIFPPSDEQLKSGTASVVCLLNNFYPREAKVQWKVDNALQSGNSQESVTEQDSKDSTYSLSSTLTLSKADYEKHKVYACEVTHQGLSSPVTKSFNRGEC

SEQ ID NO: 83 - protein, 468 aa, Homo sapiens
MDWTWRILFLVAAATGAHSEVQLVQSGAEVKKPGASVKVSCKASGYTFTDYNMHWVRQAPGQGLEWMGEINPNSGGAGYNQKFKGRVTMTTDTSTSTAYMELRSLRSDDTAVYYCARLGYDDIYDDWYFDVWGQGTTVTVSSASTKGPSVFPLAPCSRSTSESTAALGCLVKDYFPEPVTVSWNSGALTSGVHTFPAVLQSSGLYSLSSVVTVPSSNFGTQTYTCNVDHKPSNTKVDKTVERKCCVECPPCPAPPVAGPSVFLFPPKPKDTLMISRTPEVTCVVVDVSHEDPEVQFNWYVDGVEVHNAKTKPREEQFNSTFRVVSVLTVVHQDWLNGKEYKCKVSNKGLPAPIEKTISKTKGQPREPQVYTLPPSREEMTKNQVSLTCLVKGFYPSDIAVEWESNGQPENNYKTTPPMLDSDGSFFLYSKLTVDKSRWQQGNVFSCSVMHEALHNHYTQKSLSLSPGK

SEQ ID NO: 84 - protein, 240 aa, Homo sapiens
MVLQTQVFISLLLWISGAYGDIVMTQSPDSLAVSLGERATINCKSSQSVLDSSDNKNYLAWYQQKPGQPPKLLIYWASNRESGVPDRFSGSGSGTDFTLTISSLQAEDVAVYYCQQYYSDPFTFGPGTKVDIKRTVAAPSVFIFPPSDEQLKSGTASVVCLLNNFYPREAKVQWKVDNALQSGNSQESVTEQDSKDSTYSLSSTLTLSKADYEKHKVYACEVTHQGLSSPVTKSFNRGEC

SEQ ID NO: 85 - protein, 465 aa, Homo sapiens
MDWTWSILFLVAAPTGAHSQVQLVQSGAEVKKPGASVKVSCKASGYTFTSYGISWVRQAPGQGLEWMGWISAYNGNTNYAQKLQGRVTMTTDTSTSTAYMELRSLRSDDTAVYYCARESWFGEVFFDYWGQGTLVTVSSASTKGPSVFPLAPCSRSTSESTAALGCLVKDYFPEPVTVSWNSGALTSGVHTFPAVLQSSGLYSLSSVVTVPSSNFGTQTYTCNVDHKPSNTKVDKTVERKCCVECPPCPAPPVAGPSVFLFPPKPKDTLMISRTPEVTCVVVDVSHEDPEVQFNWYVDGVEVHNAKTKPREEQFNSTFRVVSVLTVVHQDWLNGKEYKCKVSNKGLPAPIEKTISKTKGQPREPQVYTLPPSREEMTKNQVSLTCLVKGFYPSDIAVEWESNGQPENNYKTTPPMLDSDGSFFLYSKLTVDKSRWQQGNVFSCSVMHEALHNHYTQKSLSLSPGK

SEQ ID NO: 86 - protein, 236 aa, Homo sapiens
MDMRVPAQLLGLLLLWLRGARCDIQMTQSPSSVSASVGDRVTITCRASQGISSWLAWYQQKPGKAPKLLIYGASNLESGVPSRFSGSGSGTDFTLTISSLQPEDFANYYCQQANSFPWTFGQGTKVEIKRTVAAPSVFIFPPSDEQLKSGTASVVCLLNNFYPREAKVQWKVDNALQSGNSQESVTEQDSKDSTYSLSSTLTLSKADYEKHKVYACEVTHQGLSSPVTKSFNRGEC

SEQ ID NO: 87 - protein, 466 aa, Homo sapiens
MDMRVPAQLLGLLLLWLRGARCQVQLVQSGAEVKKPGASVKVSCKVSGYTLSDLSIHWVRQAPGKGLEWMGGFDPQDGETIYAQKFQGRVTMTEDTSTDTAYMELSSLKSEDTAVYYCATGSSSSWFDPWGQGTLVTVSSASTKGPSVFPLAPCSRSTSESTAALGCLVKDYFPEPVTVSWNSGALTSGVHTFPAVLQSSGLYSLSSVVTVPSSNFGTQTYTCNVDHKPSNTKVDKTVERKCCVECPPCPAPPVAGPSVFLFPPKPKDTLMISRTPEVTCVVVDVSHEDPEVQFNWYVDGVEVHNAKTKPREEQFNSTFRVVSVLTVVHQDWLNGKEYKCKVSNKGLPAPIEKTISKTKGQPREPQVYTLPPSREEMTKNQVSLTCLVKGFYPSDIAVEWESNGQPENNYKTTPPMLDSDGSFFLYSKLTVDKSRWQQGNVFSCSVMHEALHNHYTQKSLSLSPGK